European Patent Specification EP 3 438 289 B1, published August 5, 2026. Title: COMPOSITIONS, METHODS AND KITS TO DETECT ADENOVIRUS NUCLEIC ACIDS. Applicant: Gen-Probe Incorporated Ziegler, Emily L Townsend, Jessica A. The sequence listing filed with the application follows.

SEQUENCE LISTING (47 sequences)

SEQ ID NO: 1 - DNA, 23 bp, Artificial Sequence
  Synthetic Oligonucleotide
caggacgcctcggrgtayctsag

SEQ ID NO: 2 - DNA, 17 bp, Artificial Sequence
  Synthetic Oligonucleotide
ggagccacvgtgggrtt

SEQ ID NO: 3 - DNA, 17 bp, Artificial Sequence
  Synthetic Oligonucleotide
aaycccacbgtggctcc

SEQ ID NO: 4 - DNA, 24 bp, Artificial Sequence
  Synthetic Oligonucleotide
ccgggtctggtgcagtttgcccgc

SEQ ID NO: 5 - DNA, 17 bp, Artificial Sequence
  Synthetic Oligonucleotide
cacatcgccggacagga

SEQ ID NO: 6 - DNA, 21 bp, Artificial Sequence
  Synthetic Oligonucleotide
catactgaagtaggtgtctgt

SEQ ID NO: 7 - DNA, 21 bp, Artificial Sequence
  Synthetic Oligonucleotide
acagacacctacttcagtatg

SEQ ID NO: 8 - DNA, 17 bp, Artificial Sequence
  Synthetic Oligonucleotide
cggtggtcacatcgtgg

SEQ ID NO: 9 - DNA, 17 bp, Artificial Sequence
  Synthetic Oligonucleotide
ccacgatgtgaccaccg

SEQ ID NO: 10 - DNA, 23 bp, Artificial Sequence
  Synthetic Oligonucleotide
agtacctcagtccgggtctggtg

SEQ ID NO: 11 - DNA, 18 bp, Artificial Sequence
  Synthetic Oligonucleotide
atggctaccccttcgatg

SEQ ID NO: 12 - DNA, 17 bp, Artificial Sequence
  Synthetic Oligonucleotide
accccmtcgatgatgcc

SEQ ID NO: 13 - DNA, 17 bp, Artificial Sequence
  Synthetic Oligonucleotide
gcgggcgaattgcacca

SEQ ID NO: 14 - DNA, 17 bp, Artificial Sequence
  Synthetic Oligonucleotide
tggtgcaattcgcccgc

SEQ ID NO: 15 - DNA, 17 bp, Artificial Sequence
  Synthetic Oligonucleotide
gcgggcaaaytgcacca

SEQ ID NO: 16 - DNA, 17 bp, Artificial Sequence
  Synthetic Oligonucleotide
tggtgcartttgcccgc

SEQ ID NO: 17 - DNA, 24 bp, Artificial Sequence
  Synthetic Oligonucleotide
gactcaggtactccgaagcatcct

SEQ ID NO: 18 - DNA, 24 bp, Artificial Sequence
  Synthetic Oligonucleotide
aggatgcttcggagtacctgagtc

SEQ ID NO: 19 - DNA, 22 bp, Artificial Sequence
  Synthetic Oligonucleotide
ctcaggtactccgaggcgtcct

SEQ ID NO: 20 - DNA, 22 bp, Artificial Sequence
  Synthetic Oligonucleotide
aggacgcctcggagtacctgag

SEQ ID NO: 21 - DNA, 22 bp, Artificial Sequence
  Synthetic Oligonucleotide
ctcaggtactccgaagcatcct

SEQ ID NO: 22 - DNA, 22 bp, Artificial Sequence
  Synthetic Oligonucleotide
aggatgcttcggagtacctgag

SEQ ID NO: 23 - DNA, 20 bp, Artificial Sequence
  Synthetic Oligonucleotide
caggtactccgaggcgtcct

SEQ ID NO: 24 - DNA, 20 bp, Artificial Sequence
  Synthetic Oligonucleotide
aggacgcctcggagtacctg

SEQ ID NO: 25 - DNA, 17 bp, Artificial Sequence
  Synthetic Oligonucleotide
accccatcgatgatgcc

SEQ ID NO: 26 - DNA, 17 bp, Artificial Sequence
  Synthetic Oligonucleotide
accccctcgatgatgcc

SEQ ID NO: 27 - DNA, 17 bp, Artificial Sequence
  Synthetic Oligonucleotide
gcgggcaaactgcacca

SEQ ID NO: 28 - DNA, 17 bp, Artificial Sequence
  Synthetic Oligonucleotide
gcgggcaaattgcacca

SEQ ID NO: 29 - DNA, 22 bp, Artificial Sequence
  Synthetic Oligonucleotide
ctcaggtattccgaggcatcct

SEQ ID NO: 30 - DNA, 22 bp, Artificial Sequence
  Synthetic Oligonucleotide
aggatgcctcggaatacctgag

SEQ ID NO: 31 - DNA, 17 bp, Artificial Sequence
  Synthetic Oligonucleotide
accccatcgatgctgcc

SEQ ID NO: 32 - DNA, 17 bp, Artificial Sequence
  Synthetic Oligonucleotide
accccatcgatgatgcc

SEQ ID NO: 33 - DNA, 18 bp, Artificial Sequence
  Synthetic Oligonucleotide
tgggcgtacatgcacatc

SEQ ID NO: 34 - DNA, 19 bp, Artificial Sequence
  Synthetic Oligonucleotide
gtggtcttacatgcacatc

SEQ ID NO: 35 - DNA, 19 bp, Artificial Sequence
  Synthetic Oligonucleotide
gtgggcatacatgcacatc

SEQ ID NO: 36 - DNA, 22 bp, Artificial Sequence
  Synthetic Oligonucleotide
aggatgcttcggagtacctgag

SEQ ID NO: 37 - DNA, 20 bp, Artificial Sequence
  Synthetic Oligonucleotide
aggacgcctcggagtacctg

SEQ ID NO: 38 - DNA, 20 bp, Artificial Sequence
  Synthetic Oligonucleotide
artggkcdtacatgcacatc

SEQ ID NO: 39 - DNA, 20 bp, Artificial Sequence
  Synthetic Oligonucleotide
caggacgcctcggagtacct

SEQ ID NO: 40 - DNA, 22 bp, Artificial Sequence
  Synthetic Oligonucleotide
aggatgcttcggagtacctgag

SEQ ID NO: 41 - DNA, 17 bp, Artificial Sequence
  Synthetic Oligonucleotide
cacgatgtgaccacaga

SEQ ID NO: 42 - DNA, 17 bp, Artificial Sequence
  Synthetic Oligonucleotide
caygatgtgaccacaga

SEQ ID NO: 43 - DNA, 17 bp, Artificial Sequence
  Synthetic Oligonucleotide
cacgaygtgaccacaga

SEQ ID NO: 44 - DNA, 17 bp, Artificial Sequence
  Synthetic Oligonucleotide
cacgatgtgaccacsga

SEQ ID NO: 45 - DNA, 17 bp, Artificial Sequence
  Synthetic Oligonucleotide
cacgatgtgaccacvga

SEQ ID NO: 46 - DNA, 17 bp, Artificial Sequence
  Synthetic Oligonucleotide
caygaygtgaccacvga

SEQ ID NO: 47 - DNA, 2832 bp, Human adenovirus 9 gene for hexon
atggccaccccctcgatgatgccgcagtgggcgtacatgcacatcgccgggcaggacgcctcggagtacctgagcccgggtctggtgcagtttgcccgcgccaccgacacgtacttcagcctgggcaacaagtttaggaaccccacggtggccccgacccacgatgtgaccacggaccggtcccagcgtctgacgctgcgcttcgtgcccgtggatcgcgaggacaccacgtactcgtacaaggcgcgcttcactctggccgtgggcgacaaccgggtgctagacatggccagcacttactttgacatccgcggcgtcctggaccgcggtcccagcttcaaaccctactcgggcacagcttacaacagtctggcccccaagggtgcccccaactccagccagtggcttgcaaaagacaccaatgctggcgatcaagcattaaaaacccacacacatggcgtagctgctatggggggaacagatatcacagcaaagggtttgcaaattggtgttgacacgactgaaaacaagaatgagcctatttatgcaaatgaaatataccagccagaacctcaggtaggagaggaaaacttgcaagatgttgaaaacttttatggaggcagagctcttaaaaaagaaaccaaaatgaaaccttgctatggctcgtttgccagacccacaaatgaaaaaggcggtcaagccaaatttttaactgacggcgatggtcagctaactaaaaatcatgatatcacaatgaatttctttgacactcctggaggaacagttggtcaggatactgaacttgaagcagacattgttatgtatgctgagaatgtgcatctggaaactccagacacgcatgtggtgtacaaaccaggaacttctgatgagagttcagaagcaaatttggttcagcagtccatgccaaacaggcccaactacatcggcttcagggacaactttgtgggtctcatgtactataacagcactggcaacatgggtgtgctggctggtcaagcatctcagttgaatgctgtggtcgacttgcaagacagaaacacagagctgtcttaccagctcttgctagattctctgggtgacagaaccagatactttagcatgtggaactctgcagtggacagttatgatcctgatgtcaggattattgaaaatcacggtgtggaagatgaacttccaaactattgcttcccattggatggagctggcactaatgctacctaccaaggtgtaaaagttaaaaatggccaagatggagatgtaaacgcagattgggaaaaagatccaaatcttgcttcacgaaaccaaatatgcaagggtaacatcttcgccatggagatcaacctccaggccaacctgtggaagagttttctgtactcgaatgtggccctgtacctgcccgactcatacaagtacacgccggccaacgtcacgctgcccgccaataccaacacctacgagtacatgaacggccgcgtggtagccccctcgctggtggacgcctacatcaacatcggcgcccggtggtcgctggaccccatggacaacgtcaacccattcaaccaccaccgcaacgcgggcctgcgttaccgctccatgcttctgggcaacggccgctacgtgcccttccacatccaagtgccccaaaagttctttgccatcaagaacctgctcctgctccccggctcctacacctacgagtggaacttccgcaaggatgtcaacatgatcctgcagagttccctcggaaacgacctgcgcgtcgacggcgcctccgtccgcttcgacagcgtcaacctctacgccacattcttccccatggcgcacaacaccgcctccaccctggaagccatgctgcgcaacgacaccaacgaccagtccttcaacgactacctctcggccgccaacatgctctaccccatcccggccaaggccaccaacgtgcccatctccatcccctcgcgcaactgggccgccttccgcggctggagtttcacccggctcaagaccaaagaaactccctccctcggctcgggtttcgatccctactttgtatactcgggttccatcccctacctcgacgggaccttctacctcaaccacaccttcaagaaggtctccatcatgttcgactcctcggtcagctggcccggcaacgaccggctgctcacgccgaacgagttcgagatcaagcgcagtgtcgacggggagggctacaatgtggcccaatgcaacatgaccaaggactggttcctcgtccagatgctctcccactacaacatcggctaccagggcttccacgtgcccgagggctacaaggaccgcatgtactccttcttccgcaacttccagcccatgagcaggcaggtggtcgatgagatcaactacaaggactacaaggccgtcaccctgcccttccagcacaacaactcgggcttcaccggctaccttgcacccaccatgcgtcaggggcagccctaccccgccaacttcccctatcctctcatcggccagacagccgtgccctctgtcacccagaaaaagttcctctgcgacagggtcatgtggcgcatccccttctccagcaacttcatgtccatgggcgccctcaccgacctgggtcagaacatgctctatgccaactcggcccacgcgctcgacatgaccttcgaggtggaccccatggatgagcccaccctcctctatcttctcttcgaagttttcgacgtggtcagagtgcaccagccgcaccgcggcgtcatcgaggccgtctacctgcgcacgcccttctccgccggcaacgccaccacctaa